European Patent Application EP 4 471 142 A1, published December 4, 2024. Title: RECOMBINANT MICROORGANISM FOR PRODUCING THREONINE AND USE THEREOF. Applicant: Langfang Meihua Biotechnology Development Co.,Ltd. Application EP 22923647.6, filed December 29, 2022. The sequence listing filed with the application follows.

SEQUENCE LISTING (50 sequences)

SEQ ID NO: 1 - protein, 919 aa, Corynebacterium glutamicum
MTDFLRDDIRFLGQILGEVIAEQEGQEVYELVEQARLTSFDIAKGNAEMDSLVQVFDGITPAKATPIARAFSHFALLANLAEDLYDEELREQALDAGDTPPDSTLDATWLKLNEGNVGAEAVADVLRNAEVAPVLTAHPTETRRRTVFDAQKWITTHMRERHALQSAEPTARTQSKLDEIEKNIRRRITILWQTALIRVARPRIEDEIEVGLRYYKLSLLEEIPRINRDVAVELRERFGEGVPLKPVVKPGSWIGGDHDGNPYVTAETVEYSTHRAAETVLKYYARQLHSLEHELSLSDRMNKVTPQLLALADAGHNDVPSRVDEPYRRAVHGVRGRILATTAELIGEDAVEGVWFKVFTPYASPEEFLNDALTIDHSLRESKDVLIADDRLSVLISAIESFGFNLYALDLRQNSESYEDVLTELFERAQVTANYRELSEAEKLEVLLKELRSPRPLIPHGSDEYSEVTDRELGIFRTASEAVKKFGPRMVPHCIISMASSVTDVLEPMVLLKEFGLIAANGDNPRGTVDVIPLFETIEDLQAGAGILDELWKIDLYRNYLLQRDNVQEVMLGYSDSNKDGGYFSANWALYDAELQLVELCRSAGVKLRLFHGRGGTVGRGGGPSYDAILAQPRGAVQGSVRITEQGEIISAKYGNPETARRNLEALVSATLEASLLDVSELTDHQRAYDIMSEISELSLKKYASLVHEDQGFIDYFTQSTPLQEIGSLNIGSRPSSRKQTSSVEDLRAIPWVLSWSQSRVMLPGWFGVGTALEQWIGEGEQATQRIAELQTLNESWPFFTSVLDNMAQVMSKAELRLAKLYADLIPDTEVAERVYSVIREEYFLTKKMFCVITGSDDLLDDNPLLARSVQRRYPYLLPLNVIQVEMMRRYRKGDQSEQVSRNIQLTMNGLSTALRNSG

SEQ ID NO: 2 - protein, 919 aa, Corynebacterium glutamicum
MTDFLRDDIRFLGQILGEVIAEQEGQEVYELVEQARLTSFDIAKGNAEMDSLVQVFDGITPAKATPIARAFSHFALLANLAEDLYDEELREQALDAGDTPPDSTLDATWLKLNEGNVGAEAVADVLRNAEVAPVLTAHPTETRRRTVFDAQKWITTHMRERHALQSAEPTARTQSKLDEIEKNIRRRITILWQTALIRVARPRIEDEIEVGLRYYKLSLLEEIPRINRDVAVELRERFGEGVPLKPVVKPGSWIGGDHDGNPYVTAETVEYSTHRAAETVLKYYARQLHSLEHELSLSNRMNKVTPQLLALADAGHNDVPSRVDEPYRRAVHGVRGRILATTAELIGEDAVEGVWFKVFTPYASPEEFLNDALTIDHSLRESKDVLIADDRLSVLISAIESFGFNLYALDLRQNSESYEDVLTELFERAQVTANYRELSEAEKLEVLLKELRSPRPLIPHGSDEYSEVTDRELGIFRTASEAVKKFGPRMVPHCIISMASSVTDVLEPMVLLKEFGLIAANGDNPRGTVDVIPLFETIEDLQAGAGILDELWKIDLYRNYLLQRDNVQEVMLGYSDSNKDGGYFSANWALYDAELQLVELCRSAGVKLRLFHGRGGTVGRGGGPSYDAILAQPRGAVQGSVRITEQGEIISAKYGNPETARRNLEALVSATLEASLLDVSELTDHQRAYDIMSEISELSLKKYASLVHEDQGFIDYFTQSTPLQEIGSLNIGSRPSSRKQTSSVEDLRAIPWVLSWSQSRVMLPGWFGVGTALEQWIGEGEQATQRIAELQTLNESWPFFTSVLDNMAQVMSKAELRLAKLYADLIPDTEVAERVYSVIREEYFLTKKMFCVITGSDDLLDDNPLLARSVQRRYPYLLPLNVIQVEMMRRYRKGDQSEQVSRNIQLTMNGLSTALRNSG

SEQ ID NO: 3 - DNA, 27 bp, synthetic construct
  source 1..27: mol_type = other DNA
caatgtgaaagagtgtttaaagtagtt

SEQ ID NO: 4 - DNA, 200 bp, synthetic construct
  source 1..200: mol_type = other DNA
tggccgttaccctgcgaatgtccacagggtagctggtagtttgaaaatcaacgccgttgcccttaggattcagtaactggcacattttgtaatgcgctagatctgtgtgctcagtcttccaggctgcttatcacagtgaaagcaaaaccaattcgtggctgcgaaagtcgtagccaccacgaagtccaggaggacataca

SEQ ID NO: 5 - DNA, 192 bp, synthetic construct
  source 1..192: mol_type = other DNA
tagctgccaattattccgggcttgtgacccgctacccgataaataggtcggctgaaaaatttcgttgcaatatcaacaaaaaggcctatcattgggaggtgtcgcaccaagtacttttgcgaagcgccatctgacggattttcaaaagatgtatatgctcggtgcggaaacctacgaaaggattttttaccc

SEQ ID NO: 6 - DNA, 260 bp, synthetic construct
  source 1..260: mol_type = other DNA
acctgcgtttataaagaaatgtaaacgtgatcggatcgatataaaagaaacagtttgtactcaggtttgaagcattttctccaattcgcctggcaaaaatctcaattgtcgcttacagtttttctcaacgacaggctgctaagctgctagttcggtggcctagtgagtggcgtttacttggataaaagtaatcccatgtcgtgatcagccattttgggttgtttccatagcatccaaaggtttcgtctttcgatacctat

SEQ ID NO: 7 - DNA, 46 bp, synthetic construct
  source 1..46: mol_type = other DNA
aattcgagctcggtacccggggatccagcgacaggacaagcactgg

SEQ ID NO: 8 - DNA, 40 bp, synthetic construct
  source 1..40: mol_type = other DNA
cccggaataattggcagctatgtgcacctttcgatctacg

SEQ ID NO: 9 - DNA, 40 bp, synthetic construct
  source 1..40: mol_type = other DNA
cgtagatcgaaaggtgcacatagctgccaattattccggg

SEQ ID NO: 10 - DNA, 41 bp, synthetic construct
  source 1..41: mol_type = other DNA
tttctgtacgaccagggccatgggtaaaaaatcctttcgta

SEQ ID NO: 11 - DNA, 41 bp, synthetic construct
  source 1..41: mol_type = other DNA
tacgaaaggattttttacccatggccctggtcgtacagaaa

SEQ ID NO: 12 - DNA, 42 bp, synthetic construct
  source 1..42: mol_type = other DNA
tcggaacgagggcaggtgaaggtgatgtcggtggtgccgtct

SEQ ID NO: 13 - DNA, 42 bp, synthetic construct
  source 1..42: mol_type = other DNA
agacggcaccaccgacatcaccttcacctgccctcgttccga

SEQ ID NO: 14 - DNA, 46 bp, synthetic construct
  source 1..46: mol_type = other DNA
gtaaaacgacggccagtgccaagcttagcctggtaagaggaaacgt

SEQ ID NO: 15 - DNA, 46 bp, synthetic construct
  source 1..46: mol_type = other DNA
aattcgagctcggtacccggggatccctgcgggcagatccttttga

SEQ ID NO: 16 - DNA, 40 bp, synthetic construct
  source 1..40: mol_type = other DNA
atttctttataaacgcaggtcatatctaccaaaactacgc

SEQ ID NO: 17 - DNA, 40 bp, synthetic construct
  source 1..40: mol_type = other DNA
gcgtagttttggtagatatgacctgcgtttataaagaaat

SEQ ID NO: 18 - DNA, 40 bp, synthetic construct
  source 1..40: mol_type = other DNA
gtatatctccttctgcaggaataggtatcgaaagacgaaa

SEQ ID NO: 19 - DNA, 40 bp, synthetic construct
  source 1..40: mol_type = other DNA
tttcgtctttcgatacctattcctgcagaaggagatatac

SEQ ID NO: 20 - DNA, 41 bp, synthetic construct
  source 1..41: mol_type = other DNA
tagccaattcagccaaaacccccacgcgatcttccacatcc

SEQ ID NO: 21 - DNA, 41 bp, synthetic construct
  source 1..41: mol_type = other DNA
ggatgtggaagatcgcgtgggggttttggctgaattggcta

SEQ ID NO: 22 - DNA, 46 bp, synthetic construct
  source 1..46: mol_type = other DNA
gtaaaacgacggccagtgccaagcttgctggctcttgccgtcgata

SEQ ID NO: 23 - DNA, 46 bp, synthetic construct
  source 1..46: mol_type = other DNA
attcgagctcggtacccggggatccgccgttgatcattgttcttca

SEQ ID NO: 24 - DNA, 40 bp, synthetic construct
  source 1..40: mol_type = other DNA
cccggaataattggcagctaggatataaccctatcccaag

SEQ ID NO: 25 - DNA, 40 bp, synthetic construct
  source 1..40: mol_type = other DNA
cttgggatagggttatatcctagctgccaattattccggg

SEQ ID NO: 26 - DNA, 41 bp, synthetic construct
  source 1..41: mol_type = other DNA
acgcgtcgaaatgtagtccatgggtaaaaaatcctttcgta

SEQ ID NO: 27 - DNA, 41 bp, synthetic construct
  source 1..41: mol_type = other DNA
tacgaaaggattttttacccatggactacatttcgacgcgt

SEQ ID NO: 28 - DNA, 46 bp, synthetic construct
  source 1..46: mol_type = other DNA
gtaaaacgacggccagtgccaagcttgaatacgcggattccctcgc

SEQ ID NO: 29 - DNA, 46 bp, synthetic construct
  source 1..46: mol_type = other DNA
aattcgagctcggtacccggggatcctacgtcgtcgagcagacccg

SEQ ID NO: 30 - DNA, 40 bp, synthetic construct
  source 1..40: mol_type = other DNA
cattcgcagggtaacggccaagggtgttggcgtgcatgag

SEQ ID NO: 31 - DNA, 40 bp, synthetic construct
  source 1..40: mol_type = other DNA
ctcatgcacgccaacacccttggccgttaccctgcgaatg

SEQ ID NO: 32 - DNA, 40 bp, synthetic construct
  source 1..40: mol_type = other DNA
tcgcgtaaaaaatcagtcattgtatgtcctcctggacttc

SEQ ID NO: 33 - DNA, 40 bp, synthetic construct
  source 1..40: mol_type = other DNA
gaagtccaggaggacatacaatgactgattttttacgcga

SEQ ID NO: 34 - DNA, 40 bp, synthetic construct
  source 1..40: mol_type = other DNA
gtgaccttattcatgcggttcgacaggctgagctcatgct

SEQ ID NO: 35 - DNA, 40 bp, synthetic construct
  source 1..40: mol_type = other DNA
agcatgagctcagcctgtcgaaccgcatgaataaggtcac

SEQ ID NO: 36 - DNA, 46 bp, synthetic construct
  source 1..46: mol_type = other DNA
gtaaaacgacggccagtgccaagcttggtgacttgggcgcgttcga

SEQ ID NO: 37 - DNA, 42 bp, synthetic construct
  source 1..42: mol_type = other DNA
gagctcggtacccggggatccgcagggtattgcagggactca

SEQ ID NO: 38 - DNA, 49 bp, synthetic construct
  source 1..49: mol_type = other DNA
caagcccggaataattggcagctaaactgcgtacctccgcatgtggtgg

SEQ ID NO: 39 - DNA, 25 bp, synthetic construct
  source 1..25: mol_type = other DNA
tagctgccaattattccgggcttgt

SEQ ID NO: 40 - DNA, 25 bp, synthetic construct
  source 1..25: mol_type = other DNA
gggtaaaaaatcctttcgtaggttt

SEQ ID NO: 41 - DNA, 53 bp, synthetic construct
  source 1..53: mol_type = other DNA
ggaaacctacgaaaggattttttacccatgagttcagtttcgctgcaggattt

SEQ ID NO: 42 - DNA, 41 bp, synthetic construct
  source 1..41: mol_type = other DNA
acgacggccagtgccaagcttacaccggaacaacccacatg

SEQ ID NO: 43 - DNA, 56 bp, synthetic construct
  source 1..56: mol_type = other DNA
tacgaattcgagctcggtacccggggatccagttaactccaccgaccgggtactgc

SEQ ID NO: 44 - DNA, 43 bp, synthetic construct
  source 1..43: mol_type = other DNA
aagcccggaataattggcagctatgtcttcgctggaccaagag

SEQ ID NO: 45 - DNA, 43 bp, synthetic construct
  source 1..43: mol_type = other DNA
ctcttggtccagcgaagacatagctgccaattattccgggctt

SEQ ID NO: 46 - DNA, 44 bp, synthetic construct
  source 1..44: mol_type = other DNA
gacggtgagaaataacatcaacatgggtaaaaaatcctttcgta

SEQ ID NO: 47 - DNA, 44 bp, synthetic construct
  source 1..44: mol_type = other DNA
tacgaaaggattttttacccatgttgatgttatttctcaccgtc

SEQ ID NO: 48 - DNA, 48 bp, synthetic construct
  source 1..48: mol_type = other DNA
tgcctcttttagccttttcagagggtcaccgcgaaataatcaaatgaa

SEQ ID NO: 49 - DNA, 48 bp, synthetic construct
  source 1..48: mol_type = other DNA
ttcatttgattatttcgcggtgaccctctgaaaaggctaaaagaggca

SEQ ID NO: 50 - DNA, 51 bp, synthetic construct
  source 1..51: mol_type = other DNA
gttgtaaaacgacggccagtgccaagcttaaaaggcagtccagtacaccct